European Patent Application EP 4 261 540 A1, published October 18, 2023. Title: MARKER FOR ASSISTING IN DIAGNOSIS OF NEPHROTIC SYNDROME AND USE THEREOF. Applicant: NIIGATA UNIVERSITY. The sequence listing filed with the application follows.

SEQUENCE LISTING (4 sequences)

SEQ ID NO: 1 - DNA, 20 bp, Artificial Sequence
  Synthetic nucleotides for forward primer of Ephrin-B1
ggcaagcatgagactgtgaa

SEQ ID NO: 2 - DNA, 20 bp, Artificial Sequence
  Synthetic nucleotides for reverse primer of Ephrin-B1
ccgtaagggaatgatgatgt

SEQ ID NO: 3 - DNA, 20 bp, Artificial Sequence
  Synthetic nucleotides for forward primer of Ephrin-B2
tccaacaagacgtccagagc

SEQ ID NO: 4 - DNA, 20 bp, Artificial Sequence
  Synthetic nucleotides for reverse primer of Ephrin-B2
agaacaaggtgcgagttccc